European Patent Specification EP 3 381 471 B1, published March 20, 2024. Title: PAIN TREATMENT. Applicant: THE UNIVERSITY OF MELBOURNE HAMILTON, John (US Only) COOK, Andrew (US Only). The sequence listing filed with the application follows.

SEQUENCE LISTING (46 sequences)

SEQ ID NO: 1 - protein, 140 aa, artificial
  amino acid sequence of heavy chain variable region
MELIMLFLLSGTAGVHSEVQLQQSGPELVKPGASVKISCKASGYTFTDYNIHWVKQSHGKSLDWIGYIAPYSGGTGYNQEFKNRATLTVDKSSSTAYMELRSLTSDDSAVYYCARRDRFPYYFDYWGQGTTLRVSSVSGS

SEQ ID NO: 2 - protein, 150 aa, artificial
  amino acid sequence of light chain variable region
MGFKMESQIQVFVYMLLWLSGVDGDIVMIQSQKFVSTSVGDRVNITCKASQNVGSNVAWLQQKPGQSPKTLIYSASYRSGRVPDRFTGSGSGTDFILTITTVQSEDLAEYFCQQFNRSPLTFGSGTKLELKRADAAPTVSIFPPSSKGEF

SEQ ID NO: 3 - protein, 117 aa, artificial [sequence omitted]

SEQ ID NO: 4 - protein, 105 aa, artificial
  amino acid sequence of light chain variable region
DIELTQPPSVSVAPGQTARISCSGDSIGKKYAYWYQQKPGQAPVLVIYKKRPSGIPERFSGSNSGNTATLTISGTQAEDEADYYCSAWGKGMVFGGGTKLTVLGQ

SEQ ID NO: 5 - protein, 10 aa, artificial
  amino acid sequence of Homo sapiens CDR3 (H-CDR3)
SGLIFDYWLD

SEQ ID NO: 6 - protein, 10 aa, artificial
  amino acid sequence of Homo sapiens CDR3 (H-CDR3)
SGLIIDALSP

SEQ ID NO: 7 - protein, 10 aa, artificial
  amino acid sequence of Homo sapiens CDR3 (H-CDR3)
TSLMSIYFDY

SEQ ID NO: 8 - protein, 10 aa, artificial
  amino acid sequence of Homo sapiens CDR3 (H-CDR3)
SGLLFLYFDY

SEQ ID NO: 9 - protein, 10 aa, artificial
  amino acid sequence of Homo sapiens CDR3 (H-CDR3)
SGLINLGMHP

SEQ ID NO: 10 - protein, 10 aa, artificial
  amino acid sequence of Homo sapiens CDR3 (H-CDR3)
SGLIFDALRD

SEQ ID NO: 11 - protein, 10 aa, artificial
  amino acid sequence of Homo sapiens CDR3 (H-CDR3)
SGLIFDKLTS

SEQ ID NO: 12 - protein, 10 aa, artificial
  amino acid sequence of Homo sapien sCDR3 (H-CDR3)
SGLINLHFDT

SEQ ID NO: 13 - protein, 10 aa, artificial
  amino acid sequence of Homo sapiens CDR3 (H-CDR3)
STHFSAYFDY

SEQ ID NO: 14 - protein, 10 aa, artificial
  amino acid sequence of Homo sapien sCDR3 (H-CDR3)
SGLIMDKLDN

SEQ ID NO: 15 - protein, 10 aa, artificial
  amino acid sequence of Homo sapiens CDR3 (H-CDR3)
SGLIIDNLNP

SEQ ID NO: 16 - protein, 10 aa, artificial
  amino acid sequence of Homo sapiens CDR3 (H-CDR3)
SGLIAVYFDY

SEQ ID NO: 17 - protein, 5 aa, artificial
  amino acid sequence of heavy CDR1 (H-CDR1)
DYLLH

SEQ ID NO: 18 - protein, 17 aa, artificial
  amino acid sequence of heavy CDR2 (H-CDR2)
WLNPYSGDTNYAQKFQG

SEQ ID NO: 19 - protein, 11 aa, artificial
  amino acid sequence of light CDR1 (L-CDR1)
RASQNIRNILN

SEQ ID NO: 20 - protein, 7 aa, artificial
  amino acid sequence fo light CDR2 (L-CDR2)
AASNLQS

SEQ ID NO: 21 - protein, 9 aa, artificial
  amino acid sequence of light CDR3 (L-CDR3)
QQSYSMPRT

SEQ ID NO: 22 - protein, 12 aa, artificial
  amino acid sequence of light CDR1 (L-CDR1)
RASHRVSSNYLA

SEQ ID NO: 23 - protein, 7 aa, artificial
  amino acid sequence of light CDR2 (L-CDR2)
GASNRAT

SEQ ID NO: 24 - protein, 9 aa, artificial
  amino acid sequence of light CDR3 (L-CDR3)
QQYASSPVT

SEQ ID NO: 25 - protein, 10 aa, artificial
  amino acid sequence of heavy CDR3 (H-CDR3)
GYIFPTFALH

SEQ ID NO: 26 - protein, 16 aa, artificial
  amino acid sequence of heavy CDR2 (H-CDR2)
SINTASGKTKFSTKFQ

SEQ ID NO: 27 - protein, 13 aa, artificial
  amino acid sequence of heavy CDR3 (H-CDR3)
DRFQNIMATILDV

SEQ ID NO: 28 - protein, 11 aa, artificial
  amino acid sequence of heavy CDR3 (H-CDR3)
VGSFSGIAYRP

SEQ ID NO: 29 - protein, 11 aa, artificial
  amino acid sequence of heavy CDR3 (H-CDR3)
VGSFSGPALRP

SEQ ID NO: 30 - protein, 11 aa, artificial
  amino acid sequence of heavy CDR3 (H-CDR3)
VGSFSPPTYGY

SEQ ID NO: 31 - protein, 11 aa, artificial
  amino acid sequence of heavy CDR3 (H-CDR3)
VGSFSGYPYRP

SEQ ID NO: 32 - protein, 11 aa, artificial
  amino acid sequence of heavy CDR3 (H-CDR3)
VGSFSPLTLGL

SEQ ID NO: 33 - protein, 11 aa, artificial
  amino acid sequence of heavy CDR3 (H-CDR3)
VGSFSGPVYGL

SEQ ID NO: 34 - protein, 11 aa, artificial
  amino acid sequence of heavy CDR3 (H-CDR3)
VGSFSPPAYRP

SEQ ID NO: 35 - protein, 11 aa, artificial
  amino acid sequence of heavy CDR3 (H-CDR3)
VGSFSPVTYGL

SEQ ID NO: 36 - protein, 11 aa, artificial
  amino acid sequence of heavy CDR3 (H-CDR3)
VGSFSGLAYRP

SEQ ID NO: 37 - protein, 11 aa, artificial
  amino acid sequence of heavy CDR3 (H-CDR3)
VGSFSPITYGL

SEQ ID NO: 38 - protein, 11 aa, artificial
  amino acid sequence of heavy CDR3 (H-CDR3)
VGSFSGWAFDY

SEQ ID NO: 39 - protein, 11 aa, artificial
  amino acid sequence of heavy CDR3 (H-CDR3)
VGSFSGWAFDY

SEQ ID NO: 40 - protein, 11 aa, artificial
  amino acid sequence of heavy CDR3 (H-CDR3)
LGSVTAWAFDY

SEQ ID NO: 41 - protein, 11 aa, artificial
  amino acid sequence of heavy CDR3 (H-CDR3)
AGSIPGWAFDY

SEQ ID NO: 42 - protein, 11 aa, artificial
  amino acid sequence of heavy CDR3 (H-CDR3)
VGSFSPLTMGL

SEQ ID NO: 43 - protein, 11 aa, artificial
  amino acid sequence of heavy CDR3 (H-CDR3)
VGSFSPLTMGL

SEQ ID NO: 44 - protein, 11 aa, artificial
  amino acid sequence of heavy CDR3 (H-CDR3)
VGSFSGPALHL

SEQ ID NO: 45 - protein, 11 aa, artificial
  amino acid sequence of heavy CDR3 (H-CDR3)
VGSVSRITYGF

SEQ ID NO: 46 - protein, 11 aa, artificial
  amino acid sequence of heavy CDR3 (H-CDR3)
VGSFSPLTLGL